European Patent Application EP 4 332 219 A1, published March 6, 2024. Title: Cargo molecule transport domain RMAD1, variant thereof, recombinant cargo molecule and cargo molecule transport method using the same. Applicant: Remedi Co., Ltd. The sequence listing filed with the application follows.

SEQUENCE LISTING (24 sequences)

SEQ ID NO: 1 - protein, 15 aa, Homo Sapiens
CKSKRRRRRRSKRKD

SEQ ID NO: 2 - protein, 15 aa, Artificial Sequence
  cargo molecule transport domain RMAD1-1
CRSKRRRRRRSRRRD

SEQ ID NO: 3 - protein, 15 aa, Artificial Sequence
  cargo molecule transport domain RMAD1-2
CKSKKKKKKKSKRKD

SEQ ID NO: 4 - protein, 11 aa, Artificial Sequence
  cargo molecule transport domain RMAD1-3
CKSKRRRRRRS

SEQ ID NO: 5 - protein, 11 aa, Artificial Sequence
  cargo molecule transport domain RMAD1-4
CKSKRRRRSKR

SEQ ID NO: 6 - protein, 11 aa, Artificial Sequence
  cargo molecule transport domain RMAD1-6
SKRRRRSKRKD

SEQ ID NO: 7 - protein, 15 aa, Artificial Sequence
  cargo molecule transport domain RMAD1-6
YKSKRRRRRRSKRKD

SEQ ID NO: 8 - protein, 18 aa, Artificial Sequence
  cargo molecule transport domain RMAD1-7
KCKSKRRRRRRSKRKDKV

SEQ ID NO: 9 - protein, 19 aa, Artificial Sequence
  cargo molecule transport domain RMAD1-8
KCKSKRRRRRRSKRKDKVS

SEQ ID NO: 10 - protein, 19 aa, Artificial Sequence
  cargo molecule transport domain RMAD1-9
LKCKSKRRRRRRSKRKDKV

SEQ ID NO: 11 - protein, 20 aa, Artificial Sequence
  cargo molecule transport domain RMAD1-10
LKCKSKRRRRRRSKRKDKVS

SEQ ID NO: 12 - DNA, 45 bp, Homo sapiens
tgcaagtccaagaggaggaggaggcggaggtccaagcggaaagat

SEQ ID NO: 13 - DNA, 45 bp, Artificial Sequence
  polynucleotide encoding cargo molecule transport domain RMAD1-1
tgcaggtccaagaggaggaggaggcggaggtccaggcggagggat

SEQ ID NO: 14 - DNA, 45 bp, Artificial Sequence
  polynucleotide encoding cargo molecule transport domain RMAD1-2
tgcaagtccaagaagaagaagaagaagaagtccaagcggaaagat

SEQ ID NO: 15 - DNA, 33 bp, Artificial Sequence
  polynucleotide encoding cargo molecule transport domain RMAD1-3
tgcaagtccaagaggaggaggaggcggaggtcc

SEQ ID NO: 16 - DNA, 33 bp, Artificial Sequence
  polynucleotide encoding cargo molecule transport domain RMAD1-4
tgcaagtccaagaggaggcggaggtccaagcgg

SEQ ID NO: 17 - DNA, 33 bp, Artificial Sequence
  polynucleotide encoding cargo molecule transport domain RMAD1-5
tccaagaggaggcggaggtccaagcggaaagat

SEQ ID NO: 18 - DNA, 45 bp, Artificial Sequence
  polynucleotide encoding cargo molecule transport domain RMAD1-6
tataagtccaagaggaggaggaggcggaggtccaagcggaaagat

SEQ ID NO: 19 - DNA, 54 bp, Artificial Sequence
  polynucleotide encoding cargo molecule transport domain RMAD1-7
aaatgcaagtccaagaggaggaggaggcggaggtccaagcggaaagataaagta

SEQ ID NO: 20 - DNA, 57 bp, Artificial Sequence
  polynucleotide encoding cargo molecule transport domain RMAD1-8
aaatgcaagtccaagaggaggaggaggcggaggtccaagcggaaagataaagtaagc

SEQ ID NO: 21 - DNA, 57 bp, Artificial Sequence
  polynucleotide encoding cargo molecule transport domain RMAD1-9
ctcaaatgcaagtccaagaggaggaggaggcggaggtccaagcggaaagataaagta

SEQ ID NO: 22 - DNA, 60 bp, Artificial Sequence
  polynucleotide encoding cargo molecule transport domain RMAD1-10
ctcaaatgcaagtccaagaggaggaggaggcggaggtccaagcggaaagataaagtaagc

SEQ ID NO: 23 - DNA, 51 bp, Artificial Sequence
  primer
agctttgcaagtccaagaggaggaggaggcggaggtccaagcggaaagatc

SEQ ID NO: 24 - DNA, 51 bp, Artificial Sequence
  primer
tcgagatctttccgcttggacctccgcctcctcctcctcttggacttgcaa